European Patent Specification EP 3 676 388 B1, published May 21, 2025. Title: Polypeptides Having D-Psicose 3-Epimerase Activity And Polynucleotides Encoding Same. Applicant: Novozymes A/S Shen, Xinyu Deinhammer, Randall S Huffman, James R. Stallings, Kendra Hoff, Tine Salomon, Jesper Olsen, Anne G. The sequence listing filed with the application follows.

SEQUENCE LISTING (8 sequences)

SEQ ID NO: 1 - DNA, 873 bp, Unknown
  Unidentified microorganism
atgaaatacggaatctactacgcctattgggaagacaagtgggaagcggactacttcaagtacatcgagaaggtcgccaagctcggcttcgacttcctggagatcgcctgcacgccgatcaacggctattccaagcagacgctgaaggacctgcgccaggcggcgaaggacaacggcatcttcctgacggccggtcacggaccgaacgccgaccagaaccttgcctcgccggacgcggctgtccgcaagaacgcgaagaagttcttcacgacgcttctcaagaacctcgagatcctcgacatccactcgatcggcggcggcatctacagctactggccggtggactactcgaagccgatcgacaagaagggcgactgggcgcgctccgtgaagggcgtgcgcgagatgggcaaggtggctcaggactgcggcgtcgactactgcctggaggtcctgaaccgcttcgagggttatctgctcaacacggccgccgaaggcgtgaagttcgtgaaagaggtggacgtgccgtccgtcaaggtcatgctcgatacgttccacatgaacatcgaggaggactcgatcggcggagcgattcgctcgaccaaggggctgctcggccacttccacacgggcgagtgcaaccgtcgcgtgccgggccgcggccgcacgccgtggcacgagatcgcctgcgcgctcaaggacatcggctacaagggcaacgtctgcatggagccgttcgttcggatgggcggcaaggtcggcgaggacatcaaggtctggcgcgaactcgaacccggcatttccgaggcgaagatggatgcggacgcgaaggcggcgctcgacttcgagaggatcgtgatggagaaggtttga

SEQ ID NO: 2 - protein, 290 aa, Unknown
  Unidentified microorganism
MKYGIYYAYWEDKWEADYFKYIEKVAKLGFDFLEIACTPINGYSKQTLKDLRQAAKDNGIFLTAGHGPNADQNLASPDAAVRKNAKKFFTTLLKNLEILDIHSIGGGIYSYWPVDYSKPIDKKGDWARSVKGVREMGKVAQDCGVDYCLEVLNRFEGYLLNTAAEGVKFVKEVDVPSVKVMLDTFHMNIEEDSIGGAIRSTKGLLGHFHTGECNRRVPGRGRTPWHEIACALKDIGYKGNVCMEPFVRMGGKVGEDIKVWRELEPGISEAKMDADAKAALDFERIVMEKV

SEQ ID NO: 3 - DNA, 870 bp, Unknown
  Unidentified microorganism
atgaagtttggaacctattttgcctattgggaaaaagactgggatacggattatattaagtatgtaaaaaaagttgccgacctgggctttgatgttttagaagtaggagctgcagggattgttaatatgtctgatgaacaattatttgctttaaagtctgaagcggagaaattcaatattactttaacagccgggattggtcttccgaaggaatatgatgtttcttctctagatgaagatgtccgacagaatggaattgcttttatgaaaagaattttagacgcattatataaagccggcatacatgcaatcggcggaacaatctattcttattggcctgccgattatacttctcctataaacaaaccagaagttcgaaaacaaagcattaaaagtatgaaagaattggctgattatgcagctcagtataatatcactttgctggtggaaacactaaaccgatttgagcagtttttaattaatgatgcaaaagaagctgtcgcctttgtaaaagatattaataaagagaatgttaaggtcatgttagatagttttcatatgaacattgaggaagattatattggggatgcgatccgctatacaggtgaatatttagggcatttccatatcggagaatgcaatcgcaaagtgcctggcaaaggtcatatgccttgggcagaaattggacaggctcttcgggatattaattacaatggatgcgtcgtcatggaaccatttgttcgtacaggtggggttgtaggatcagatataagagtctggagagatctttccgaaaatgcagatgatgctaaattagatgcagatattaaagaatctcttgaatttattaaaaacgagtttttaaaatag

SEQ ID NO: 4 - protein, 289 aa, Unknown
  Unidentified microorganism
MKFGTYFAYWEKDWDTDYIKYVKKVADLGFDVLEVGAAGIVNMSDEQLFALKSEAEKFNITLTAGIGLPKEYDVSSLDEDVRQNGIAFMKRILDALYKAGIHAIGGTIYSYWPADYTSPINKPEVRKQSIKSMKELADYAAQYNITLLVETLNRFEQFLINDAKEAVAFVKDINKENVKVMLDSFHMNIEEDYIGDAIRYTGEYLGHFHIGECNRKVPGKGHMPWAEIGQALRDINYNGCVVMEPFVRTGGVVGSDIRVWRDLSENADDAKLDADIKESLEFIKNEFLK

SEQ ID NO: 5 - DNA, 870 bp, Artificial Sequence
  Artificial DNA Sequence
atgaagtatggcatctactatgcatactgggaggacaaatgggaggctgactatttcaaatacatcgagaaagttgcaaaacttggtttcgacttccttgagatcgcgtgcacaccaatcaacggatattctaaacaaactcttaaggaccttcgccaagctgcgaaagacaacggcatctttcttactgctggccatggtccgaacgctgaccaaaaccttgcttctccggacgcagctgttcgcaaaaacgcgaagaaattcttcacgacacttcttaagaaccttgagatcttagacatccactctatcggtggcggaatctattcatactggcctgttgactactctaaacctatcgacaaaaagggcgactgggctcgctctgttaaaggcgtacgcgagatgggcaaagtagctcaagactgtggcgttgactattgccttgaggtacttaaccgcttcgagggctaccttcttaacactgcagctgagggcgttaagtttgttaaagaggttgacgtaccatctgttaaagttatgttagacacattccacatgaacatcgaggaggactctattggtggcgcaatccgctcaactaagggccttcttggccattttcatactggcgagtgtaatcgtcgcgttcctggtcgtggtcgcactccatggcatgagatcgcttgcgctcttaaagacatcggctacaaaggcaacgtttgtatggagccttttgtacgcatgggtggcaaagttggcgaggacatcaaagtttggcgtgagcttgagcctggcatctctgaggccaaaatggacgcagacgcaaaagcagctcttgacttcgagcgcatcgttatggagaaggta

SEQ ID NO: 6 - DNA, 867 bp, Artificial Sequence
  Artificial DNA Sequence
atgaaattcggcacttacttcgcttactgggagaaggactgggacacggactacatcaagtacgtaaagaaggttgctgaccttggcttcgacgttcttgaggtaggcgctgcaggcatcgttaacatgagcgacgagcaacttttcgcacttaagtctgaggctgagaagttcaacatcacacttacagctggcatcggccttcctaaggagtatgacgttagcagccttgacgaggacgtacgccagaacggcatcgctttcatgaagcgcatccttgacgcactttacaaggctggcatccacgcgattggtggcactatctactcttattggcctgcagactacacatctcctatcaacaaacctgaggtacgcaaacaatcaatcaagtctatgaaggagcttgctgactatgctgctcaatacaacatcactcttcttgttgagactcttaaccgctttgagcagtttcttatcaacgacgcaaaggaggctgttgcgttcgtaaaggacatcaacaaggagaacgttaaggttatgcttgactctttccacatgaacatcgaggaggactacatcggcgacgcaatccgctacactggcgagtaccttggccacttccatatcggcgagtgtaaccgcaaagttccaggcaagggccatatgccttgggcagagatcggccaagcgcttcgcgacatcaactataacggctgcgttgttatggagccatttgttcgcactggtggcgtagtaggcagcgacatccgcgtatggcgtgaccttagcgagaacgcggacgacgctaagcttgacgctgacatcaaggagtcacttgagttcatcaagaacgagttccttaag

SEQ ID NO: 7 - DNA, 29 bp, Artificial Sequence
  Artificial Primer
gagctctataaaaatgaggagggaaccga

SEQ ID NO: 8 - DNA, 27 bp, Artificial Sequence
  Artificial Primer
catcatcaccatcaccactaaacgcgt